European Patent Specification EP 3 153 524 B1, published April 23, 2025. Title: ANTIBODY VARIANTS HAVING MODIFICATIONS IN THE CONSTANT REGION. Applicant: Genmab A/S. The sequence listing filed with the application follows.

SEQUENCE LISTING (9 sequences)

SEQ ID NO: 1 - DNA, 1588 bp, Homo sapiens
gctagcaccaagggcccatccgtcttccccctggcgccctgctccaggagcacctccgagagcacagccgccctgggctgcctggtcaaggactacttccccgaaccggtgacggtgtcgtggaactcaggcgccctgaccagcggcgtgcacaccttcccggctgtcctacagtcctcaggactctactccctcagcagcgtggtgaccgtgccctccagcagcttgggcacgaagacctacacctgcaacgtagatcacaagcccagcaacaccaaggtggacaagagagttggtgagaggccagcacagggagggagggtgtctgctggaagccaggctcagccctcctgcctggacgcaccccggctgtgcagccccagcccagggcagcaaggcatgccccatctgtctcctcacccggaggcctctgaccaccccactcatgctcagggagagggtcttctggatttttccaccaggctccgggcagccacaggctggatgcccctaccccaggccctgcgcatacaggggcaggtgctgcgctcagacctgccaagagccatatccgggaggaccctgcccctgacctaagcccaccccaaaggccaaactctccactccctcagctcagacaccttctctcctcccagatctgagtaactcccaatcttctctctgcagagtccaaatatggtcccccatgcccatcatgcccaggtaagccaacccaggcctcgccctccagctcaaggcgggacaggtgccctagagtagcctgcatccagggacaggccccagccgggtgctgacgcatccacctccatctcttcctcagcacctgagttcctggggggaccatcagtcttcctgttccccccaaaacccaaggacactctcatgatctcccggacccctgaggtcacgtgcgtggtggtggacgtgagccaggaagaccccgaggtccagttcaactggtacgtggatggcgtggaggtgcataatgccaagacaaagccgcgggaggagcagttcaacagcacgtaccgtgtggtcagcgtcctcaccgtcctgcaccaggactggctgaacggcaaggagtacaagtgcaaggtctccaacaaaggcctcccgtcctccatcgagaaaaccatctccaaagccaaaggtgggacccacggggtgcgagggccacatggacagaggtcagctcggcccaccctctgccctgggagtgaccgctgtgccaacctctgtccctacagggcagccccgagagccacaggtgtacaccctgcccccatcccaggaggagatgaccaagaaccaggtcagcctgacctgcctggtcaaaggcttctaccccagcgacatcgccgtggagtgggagagcaatgggcagccggagaacaactacaagaccacgcctcccgtgctggactccgacggctccttcttcctctacagcaggctaaccgtggacaagagcaggtggcaggaggggaatgtcttctcatgctccgtgatgcatgaggctctgcacaaccactacacacagaagagcctctccctgtctctgggtaaa

SEQ ID NO: 2 - protein, 327 aa, Homo sapiens
  VARIANT (189)..(189): X at position 189 is Leu or Val
  VARIANT (289)..(289): X at position 289 is Arg or Lysl
ASTKGPSVFPLAPCSRSTSESTAALGCLVKDYFPEPVTVSWNSGALTSGVHTFPAVLQSSGLYSLSSVVTVPSSSLGTKTYTCNVDHKPSNTKVDKRVESKYGPPCPSCPAPEFLGGPSVFLFPPKPKDTLMISRTPEVTCVVVDVSQEDPEVQFNWYVDGVEVHNAKTKPREEQFNSTYRVVSVLTVXHQDWLNGKEYKCKVSNKGLPSSIEKTISKAKGQPREPQVYTLPPSQEEMTKNQVSLTCLVKGFYPSDIAVEWESNGQPENNYKTTPPVLDSDGSFFLYSXLTVDKSRWQEGNVFSCSVMHEALHNHYTQKSLSLSLGK

SEQ ID NO: 3 - DNA, 1588 bp, Homo sapiens
gctagcaccaagggcccatccgtcttccccctggcgccctgctccaggagcacctccgagagcacagccgccctgggctgcctggtcaaggactacttccccgaaccggtgacggtgtcgtggaactcaggcgccctgaccagcggcgtgcacaccttcccggctgtcctacagtcctcaggactctactccctcagcagcgtggtgaccgtgccctccagcagcttgggcacgaagacctacacctgcaacgtagatcacaagcccagcaacaccaaggtggacaagagagttggtgagaggccagcacagggagggagggtgtctgctggaagccaggctcagccctcctgcctggacgcaccccggctgtgcagccccagcccagggcagcaaggcatgccccatctgtctcctcacccggaggcctctgaccaccccactcatgctcagggagagggtcttctggatttttccaccaggctccgggcagccacaggctggatgcccctaccccaggccctgcgcatacaggggcaggtgctgcgctcagacctgccaagagccatatccgggaggaccctgcccctgacctaagcccaccccaaaggccaaactctccactccctcagctcagacaccttctctcctcccagatctgagtaactcccaatcttctctctgcagagtccaaatatggtcccccatgcccaccatgcccgggtaagccaacccaggcctcgccctccagctcaaggcgggacaggtgccctagagtagcctgcatccagggacaggccccagccgggtgctgacgcatccacctccatctcttcctcagcacctgagttcctggggggaccatcagtcttcctgttccccccaaaacccaaggacactctcatgatctcccggacccctgaggtcacgtgcgtggtggtggacgtgagccaggaagaccccgaggtccagttcaactggtacgtggatggcgtggaggtgcataatgccaagacaaagccgcgggaggagcagttcaacagcacgtaccgtgtggtcagcgtcctcaccgtcctgcaccaggactggctgaacggcaaggagtacaagtgcaaggtctccaacaaaggcctcccgtcctccatcgagaaaaccatctccaaagccaaaggtgggacccacggggtgcgagggccacatggacagaggtcagctcggcccaccctctgccctgggagtgaccgctgtgccaacctctgtccctacagggcagccccgagagccacaggtgtacaccctgcccccatcccaggaggagatgaccaagaaccaggtcagcctgacctgcctggtcaaaggcttctaccccagcgacatcgccgtggagtgggagagcaatgggcagccggagaacaactacaagaccacgcctcccgtgctggactccgacggctccttcttcctctacagcaggctaaccgtggacaagagcaggtggcaggaggggaatgtcttctcatgctccgtgatgcatgaggctctgcacaaccactacacacagaagagcctctccctgtctctgggtaaa

SEQ ID NO: 4 - protein, 315 aa, Homo sapiens
ASTKGPSVFPLAPCSRSTSESTAALGCLVKDYFPEPVTVSWNSGALTSGVHTFPAVLQSSGLYSLSSVVTVPSSSLGTKTYTCNVDHKPSNTKVDKRVAPEFLGGPSVFLFPPKPKDTLMISRTPEVTCVVVDVSQEDPEVQFNWYVDGVEVHNAKTKPREEQFNSTYRVVSVLTVLHQDWLNGKEYKCKVSNKGLPSSIEKTISKAKGQPREPQVYTLPPSQEEMTKNQVSLTCLVKGFYPSDIAVEWESNGQPENNYKTTPPVLDSDGSFFLYSRLTVDKSRWQEGNVFSCSVMHEALHNHYTQKSLSLSLGK

SEQ ID NO: 5 - protein, 105 aa, Homo sapiens
QPKAAPSVTLFPPSSEELQANKATLVCLISDFYPGAVTVAWKADSSPVKAGVETTTPSKQSNNKYAASSYLSLTPEQWKSHRSYSCQVTHEGSTVEKTVAPTECS

SEQ ID NO: 6 - protein, 106 aa, Homo sapiens
TVAAPSVFIFPPSDEQLKSGTASVVCLLNNFYPREAKVQWKVDNALQSGNSQESVTEQDSKDSTYSLSSTLTLSKADYEKHKVYACEVTHQGLSSPVTKSFNRGEC

SEQ ID NO: 7 - protein, 330 aa, Homo sapiens
ASTKGPSVFPLAPSSKSTSGGTAALGCLVKDYFPEPVTVSWNSGALTSGVHTFPAVLQSSGLYSLSSVVTVPSSSLGTQTYICNVNHKPSNTKVDKKVEPKSCDKTHTCPPCPAPELLGGPSVFLFPPKPKDTLMISRTPEVTCVVVDVSHEDPEVKFNWYVDGVEVHNAKTKPREEQYNSTYRVVSVLTVLHQDWLNGKEYKCKVSNKALPAPIEKTISKAKGQPREPQVYTLPPSRDEMTKNQVSLTCLVKGFYPSDIAVEWESNGQPENNYKTTPPVLDSDGSFFLYSKLTVDKSRWQQGNVFSCSVMHEALHNHYTQKSLSLSPGK

SEQ ID NO: 8 - protein, 326 aa, Homo sapiens
ASTKGPSVFPLAPCSRSTSESTAALGCLVKDYFPEPVTVSWNSGALTSGVHTFPAVLQSSGLYSLSSVVTVPSSNFGTQTYTCNVDHKPSNTKVDKTVERKCCVECPPCPAPPVAGPSVFLFPPKPKDTLMISRTPEVTCVVVDVSHEDPEVQFNWYVDGVEVHNAKTKPREEQFNSTFRVVSVLTVVHQDWLNGKEYKCKVSNKGLPAPIEKTISKTKGQPREPQVYTLPPSREEMTKNQVSLTCLVKGFYPSDIAVEWESNGQPENNYKTTPPMLDSDGSFFLYSKLTVDKSRWQQGNVFSCSVMHEALHNHYTQKSLSLSPGK

SEQ ID NO: 9 - protein, 377 aa, Homo sapiens
ASTKGPSVFPLAPCSRSTSGGTAALGCLVKDYFPEPVTVSWNSGALTSGVHTFPAVLQSSGLYSLSSVVTVPSSSLGTQTYTCNVNHKPSNTKVDKRVELKTPLGDTTHTCPRCPEPKSCDTPPPCPRCPEPKSCDTPPPCPRCPEPKSCDTPPPCPRCPAPELLGGPSVFLFPPKPKDTLMISRTPEVTCVVVDVSHEDPEVQFKWYVDGVEVHNAKTKPREEQYNSTFRVVSVLTVLHQDWLNGKEYKCKVSNKALPAPIEKTISKTKGQPREPQVYTLPPSREEMTKNQVSLTCLVKGFYPSDIAVEWESSGQPENNYNTTPPMLDSDGSFFLYSKLTVDKSRWQQGNIFSCSVMHEALHNRFTQKSLSLSPGK